European Patent Application EP 4 328 325 A1, published February 28, 2024. Title: COMPOSITION, KIT, AND APPLICATION FOR DETECTION OF COLORECTAL CANCER. Applicant: BGI GENOMICS CO., LTD. The sequence listing filed with the application follows.

SEQUENCE LISTING (142 sequences)

SEQ ID NO: 1 - DNA, 23 bp, Artificial Sequence
  GAPDH forward primer 1
tttaggagtgagtggaagataga

SEQ ID NO: 2 - DNA, 23 bp, Artificial Sequence
  GAPDH reverse primer 1
aaaccacaccatcctaattacct

SEQ ID NO: 3 - DNA, 17 bp, Artificial Sequence
  ADHFE1 forward primer 1
tcgttggggtagttggc

SEQ ID NO: 4 - DNA, 24 bp, Artificial Sequence
  ADHFE1 reverse primer 1
cctatctaaacctcaaaccaatcg

SEQ ID NO: 5 - DNA, 20 bp, Artificial Sequence
  ADHFE1 forward primer 2
gttttgggtttttatcgcgc

SEQ ID NO: 6 - DNA, 21 bp, Artificial Sequence
  ADHFE1 reverse primer 2
gccctaaaaaactacatcgcg

SEQ ID NO: 7 - DNA, 15 bp, Artificial Sequence
  ADHFE1 forward primer 3
gatggtgcgagcgtc

SEQ ID NO: 8 - DNA, 23 bp, Artificial Sequence
  ADHFE1 reverse primer 3
ctatctaaacctcaaaccaatcg

SEQ ID NO: 9 - DNA, 20 bp, Artificial Sequence
  ADHFE1 forward primer 4
ggtaattttaagggtggatg

SEQ ID NO: 10 - DNA, 19 bp, Artificial Sequence
  ADHFE1 reverse primer 4
ctcaaaaccattttcccac

SEQ ID NO: 11 - DNA, 21 bp, Artificial Sequence
  ADHFE1 forward primer 5
aagtaaggagatttaaggtag

SEQ ID NO: 12 - DNA, 19 bp, Artificial Sequence
  ADHFE1 reverse primer 5
ctcaaaaccattttcccac

SEQ ID NO: 13 - DNA, 24 bp, Artificial Sequence
  ADHFE1 forward primer 6
gggttatttgtttaagttttaagt

SEQ ID NO: 14 - DNA, 16 bp, Artificial Sequence
  ADHFE1 reverse primer 6
ccccaaatcctcaaca

SEQ ID NO: 15 - DNA, 21 bp, Artificial Sequence
  ADHFE1 forward primer 7
gttgtagttgttttagtaagt

SEQ ID NO: 16 - DNA, 22 bp, Artificial Sequence
  ADHFE1 reverse primer 7
ttaaaacttaaacaaataaccc

SEQ ID NO: 17 - DNA, 19 bp, Artificial Sequence
  ADHFE1 forward primer 8
gattggtttgaggtttaga

SEQ ID NO: 18 - DNA, 16 bp, Artificial Sequence
  ADHFE1 reverse primer 8
aatcctcttccctcct

SEQ ID NO: 19 - DNA, 19 bp, Artificial Sequence
  ADHFE1 forward primer 9
gattggtttgaggtttaga

SEQ ID NO: 20 - DNA, 22 bp, Artificial Sequence
  ADHFE1 reverse primer 9
ttacaattacctcaacaaatac

SEQ ID NO: 21 - DNA, 23 bp, Artificial Sequence
  ADHFE1 forward primer 10
ggtaattttaagggtggatggtg

SEQ ID NO: 22 - DNA, 23 bp, Artificial Sequence
  ADHFE1 reverse primer 10
tcacctatctaaacctcaaacca

SEQ ID NO: 23 - DNA, 22 bp, Artificial Sequence
  ADHFE1 forward primer 11
aggtttagataggtgatttcgc

SEQ ID NO: 24 - DNA, 16 bp, Artificial Sequence
  ADHFE1 reverse primer 11
aaactacccgcctccc

SEQ ID NO: 25 - DNA, 22 bp, Artificial Sequence
  ADHFE1 forward primer 12
ttggcgttttggtttttatttc

SEQ ID NO: 26 - DNA, 24 bp, Artificial Sequence
  ADHFE1 reverse primer 12
cctatctaaacctcaaaccaatcg

SEQ ID NO: 27 - DNA, 26 bp, Artificial Sequence
  ADHFE1 forward primer 13
gatttaaggtagaattcgaggtttac

SEQ ID NO: 28 - DNA, 21 bp, Artificial Sequence
  ADHFE1 reverse primer 13
cacgaaataaaaaccaaaacg

SEQ ID NO: 29 - DNA, 22 bp, Artificial Sequence
  ADHFE1 forward primer 14
cgtagttttttgggtgtgattc

SEQ ID NO: 30 - DNA, 22 bp, Artificial Sequence
  ADHFE1 reverse primer 14
aaaacgatatccaaattctccg

SEQ ID NO: 31 - DNA, 24 bp, Artificial Sequence
  ADHFE1 forward primer 15
cgtattttgtgatttcgttgtttc

SEQ ID NO: 32 - DNA, 25 bp, Artificial Sequence
  ADHFE1 reverse primer 15
aaaaattcgaaaaatttaaataccg

SEQ ID NO: 33 - DNA, 20 bp, Artificial Sequence
  ADHFE1 forward primer 16
cgtttgtttattcgtttcgc

SEQ ID NO: 34 - DNA, 20 bp, Artificial Sequence
  ADHFE1 reverse primer 16
cgccgctaaaacaactaacg

SEQ ID NO: 35 - DNA, 21 bp, Artificial Sequence
  ADHFE1 forward primer 17
cgttttgagaggttgtatcgc

SEQ ID NO: 36 - DNA, 25 bp, Artificial Sequence
  ADHFE1 reverse primer 17
aaaaattcgaaaaatttaaataccg

SEQ ID NO: 37 - DNA, 25 bp, Artificial Sequence
  ADHFE1 forward primer 18
gtttagggcggtatttaaatttttc

SEQ ID NO: 38 - DNA, 23 bp, Artificial Sequence
  ADHFE1 reverse primer 18
atataacccgctcaaatcctacg

SEQ ID NO: 39 - DNA, 23 bp, Artificial Sequence
  ADHFE1 forward primer 19
tgtatcgcgtattttgtgatttc

SEQ ID NO: 40 - DNA, 21 bp, Artificial Sequence
  ADHFE1 reverse primer 19
ccgcttactttcaaaaattcg

SEQ ID NO: 41 - DNA, 20 bp, Artificial Sequence
  PPP2R5C forward primer 1
ggttttcgttgtttcgtttc

SEQ ID NO: 42 - DNA, 18 bp, Artificial Sequence
  PPP2R5C reverse primer 1
ccaaatcgacgtcctccg

SEQ ID NO: 43 - DNA, 19 bp, Artificial Sequence
  PPP2R5C forward primer 2
ggttttaggtcggggtttc

SEQ ID NO: 44 - DNA, 16 bp, Artificial Sequence
  PPP2R5C reverse primer 2
cctcctccgaactccg

SEQ ID NO: 45 - DNA, 21 bp, Artificial Sequence
  PPP2R5C forward primer 3
tttcggtatgggttttaggtc

SEQ ID NO: 46 - DNA, 16 bp, Artificial Sequence
  PPP2R5C reverse primer 3
cctcctccgaactccg

SEQ ID NO: 47 - DNA, 21 bp, Artificial Sequence
  PPP2R5C forward primer 4
cgttgtttcgtttcggagttc

SEQ ID NO: 48 - DNA, 17 bp, Artificial Sequence
  PPP2R5C reverse primer 4
caaatcgacgtcctccg

SEQ ID NO: 49 - DNA, 21 bp, Artificial Sequence
  PPP2R5C forward primer 5
tgtttcggttttcgttgtttc

SEQ ID NO: 50 - DNA, 17 bp, Artificial Sequence
  PPP2R5C reverse primer 5
caaatcgacgtcctccg

SEQ ID NO: 51 - DNA, 16 bp, Artificial Sequence
  PPP2R5C forward primer 6
ggaaacgggagagcgc

SEQ ID NO: 52 - DNA, 20 bp, Artificial Sequence
  PPP2R5C reverse primer 6
cgccgatctaacctcctacg

SEQ ID NO: 53 - DNA, 17 bp, Artificial Sequence
  PPP2R5C forward primer 7
cgggacggaaaggaaac

SEQ ID NO: 54 - DNA, 19 bp, Artificial Sequence
  PPP2R5C reverse primer 7
gccgatctaacctcctacg

SEQ ID NO: 55 - DNA, 17 bp, Artificial Sequence
  PPP2R5C forward primer 8
ggttggaggatgaagtt

SEQ ID NO: 56 - DNA, 18 bp, Artificial Sequence
  PPP2R5C reverse primer 8
tccaaccctctacttaac

SEQ ID NO: 57 - DNA, 16 bp, Artificial Sequence
  PPP2R5C forward primer 9
ggtatgggttttaggt

SEQ ID NO: 58 - DNA, 19 bp, Artificial Sequence
  PPP2R5C reverse primer 9
actaaaaaataaaaccccc

SEQ ID NO: 59 - DNA, 16 bp, Artificial Sequence
  PPP2R5C forward primer 10
aagtagagggttggag

SEQ ID NO: 60 - DNA, 16 bp, Artificial Sequence
  PPP2R5C reverse primer 10
aaaacccttaactccc

SEQ ID NO: 61 - DNA, 27 bp, Artificial Sequence
  SDC2 forward primer 1
agtgtagaaattaataagtgagagggc

SEQ ID NO: 62 - DNA, 20 bp, Artificial Sequence
  SDC2 reverse primer 1
ttcctcctcctacgcctact

SEQ ID NO: 63 - DNA, 19 bp, Artificial Sequence
  SDC2 forward primer 2
ataagtgagagggcgtcgc

SEQ ID NO: 64 - DNA, 20 bp, Artificial Sequence
  SDC2 reverse primer 2
ttcctcctcctacgcctact

SEQ ID NO: 65 - DNA, 19 bp, Artificial Sequence
  SDC2 forward primer 3
cgttgcggtattttgtttc

SEQ ID NO: 66 - DNA, 19 bp, Artificial Sequence
  SDC2 reverse primer 3
aacgaaacctcctacccaa

SEQ ID NO: 67 - DNA, 25 bp, Artificial Sequence
  SDC2 forward primer 4
aaattagaaattgaatttcggtacg

SEQ ID NO: 68 - DNA, 31 bp, Artificial Sequence
  SDC2 reverse primer 4
aactactctctaaaactcttcttactctact

SEQ ID NO: 69 - DNA, 19 bp, Artificial Sequence
  SDC2 forward primer 5
gcgttgggtaggaggtttc

SEQ ID NO: 70 - DNA, 23 bp, Artificial Sequence
  SDC2 reverse primer 5
atattccccaaaaaccgactact

SEQ ID NO: 71 - DNA, 23 bp, Artificial Sequence
  SDC2 forward primer 6
tcgtttagggtgtttgaagttac

SEQ ID NO: 72 - DNA, 24 bp, Artificial Sequence
  SDC2 reverse primer 6
ccaacgaatctccgatatatactt

SEQ ID NO: 73 - DNA, 17 bp, Artificial Sequence
  SDC2 forward primer 7
cgtggtttgggaaggac

SEQ ID NO: 74 - DNA, 20 bp, Artificial Sequence
  SDC2 reverse primer 7
cgaaataaaaccgttccctc

SEQ ID NO: 75 - DNA, 18 bp, Artificial Sequence
  SDC2 forward primer 8
ggagtttgggtcgggttc

SEQ ID NO: 76 - DNA, 25 bp, Artificial Sequence
  SDC2 reverse primer 8
aaatttccaaatcatccctaatctc

SEQ ID NO: 77 - DNA, 28 bp, Artificial Sequence
  SDC2 forward primer 9
gggagtgtagaaattaataagtgagagg

SEQ ID NO: 78 - DNA, 18 bp, Artificial Sequence
  SDC2 reverse primer 9
ctcctacgcctactcccg

SEQ ID NO: 79 - DNA, 24 bp, Artificial Sequence
  SDC2 forward primer 10
gagttcgagttttcgagtttgagt

SEQ ID NO: 80 - DNA, 17 bp, Artificial Sequence
  SDC2 reverse primer 10
ctacccaacgctcgacg

SEQ ID NO: 81 - DNA, 24 bp, Artificial Sequence
  SDC2 forward primer 11
gagttcgagttttcgagtttgagt

SEQ ID NO: 82 - DNA, 19 bp, Artificial Sequence
  SDC2 reverse primer 11
cgaaacctcctacccaacg

SEQ ID NO: 83 - DNA, 20 bp, Artificial Sequence
  SDC2 forward primer 12
gagtcggtgagtgggttagg

SEQ ID NO: 84 - DNA, 18 bp, Artificial Sequence
  SDC2 reverse primer 12
gctcccctattccctacg

SEQ ID NO: 85 - DNA, 18 bp, Artificial Sequence
  SDC2 forward primer 13
atattttaaacggcgcgc

SEQ ID NO: 86 - DNA, 31 bp, Artificial Sequence
  SDC2 reverse primer 13
taaatcctactcaccttaaacttaataacct

SEQ ID NO: 87 - DNA, 18 bp, Artificial Sequence
  SDC2 forward primer 14
ttgaggaagggaagaggg

SEQ ID NO: 88 - DNA, 20 bp, Artificial Sequence
  SDC2 reverse primer 14
caatccccaaatatacaccg

SEQ ID NO: 89 - DNA, 24 bp, Artificial Sequence
  SDC2 forward primer 15
tttagggatcggttgtttttagtc

SEQ ID NO: 90 - DNA, 22 bp, Artificial Sequence
  SDC2 reverse primer 15
gaattcgtatacgcgaactacg

SEQ ID NO: 91 - DNA, 25 bp, Artificial Sequence
  SDC2 forward primer 16
agtttaaggtgagtaggatttacgc

SEQ ID NO: 92 - DNA, 25 bp, Artificial Sequence
  SDC2 reverse primer 16
ttttaccctaattacaaacaacgac

SEQ ID NO: 93 - DNA, 23 bp, Artificial Sequence
  SDC2 forward primer 17
ggtttttgcggttagattaaatc

SEQ ID NO: 94 - DNA, 22 bp, Artificial Sequence
  SDC2 reverse primer 17
aaaaaacgctactcgctaacgt

SEQ ID NO: 95 - DNA, 16 bp, Artificial Sequence
  SDC2 forward primer 18
gtagggaataggggag

SEQ ID NO: 96 - DNA, 19 bp, Artificial Sequence
  SDC2 reverse primer 18
aaataacttcaaaaacctc

SEQ ID NO: 97 - DNA, 18 bp, Artificial Sequence
  SDC2 forward primer 19
gaagaagttgggagtgat

SEQ ID NO: 98 - DNA, 16 bp, Artificial Sequence
  SDC2 reverse primer 19
cctcttcccttcctca

SEQ ID NO: 99 - DNA, 23 bp, Artificial Sequence
  GAPDH probe 1
cccaaaacacatttcttccattc

SEQ ID NO: 100 - DNA, 24 bp, Artificial Sequence
  SDC2 probe 1
aaacgaagttttttgtttagcgtt

SEQ ID NO: 101 - DNA, 27 bp, Artificial Sequence
  SDC2 probe 2
gaaaaaacttcgttttaccctaattac

SEQ ID NO: 102 - DNA, 27 bp, Artificial Sequence
  SDC2 probe 3
acaccgaaaattacgatttaatctaac

SEQ ID NO: 103 - DNA, 27 bp, Artificial Sequence
  SDC2 probe 4
acaccaaaaattacaatttaatctaac

SEQ ID NO: 104 - DNA, 19 bp, Artificial Sequence
  SDC2 probe 5
ctactcgctaacgttaccc

SEQ ID NO: 105 - DNA, 19 bp, Artificial Sequence
  SDC2 probe 6
ctactcactaacattaccc

SEQ ID NO: 106 - DNA, 16 bp, Artificial Sequence
  SDC2 probe 7
cctcttcccttcctca

SEQ ID NO: 107 - DNA, 22 bp, Artificial Sequence
  SDC2 probe 8
taacgccaacgaacaacgcttt

SEQ ID NO: 108 - DNA, 25 bp, Artificial Sequence
  SDC2 probe 9
ctaaaccaaaccgcaattctcgata

SEQ ID NO: 109 - DNA, 22 bp, Artificial Sequence
  SDC2 probe 10
taacaccaacaaacaacacttt

SEQ ID NO: 110 - DNA, 25 bp, Artificial Sequence
  SDC2 probe 11
ctaaaccaaaccacaattctcaata

SEQ ID NO: 111 - DNA, 24 bp, Artificial Sequence
  SDC2 probe 12
accccgcgatccgcgaaaataaaa

SEQ ID NO: 112 - DNA, 28 bp, Artificial Sequence
  SDC2 probe 13
cccgcgatccgcgaaaataaaaacaccg

SEQ ID NO: 113 - DNA, 23 bp, Artificial Sequence
  ADHFE1 probe 1
tcacctatctaaacctcaaacca

SEQ ID NO: 114 - DNA, 17 bp, Artificial Sequence
  ADHFE1 probe 2
cccaacgacgctcgcac

SEQ ID NO: 115 - DNA, 18 bp, Artificial Sequence
  ADHFE1 probe 3
caacgacgctcgcaccat

SEQ ID NO: 116 - DNA, 25 bp, Artificial Sequence
  ADHFE1 probe 4
taaataatacgaacgccgctaaaac

SEQ ID NO: 117 - DNA, 26 bp, Artificial Sequence
  ADHFE1 probe 5
atacgaacgccgctaaaacaactaac

SEQ ID NO: 118 - DNA, 17 bp, Artificial Sequence
  ADHFE1 probe 6
cccaacaacactcacac

SEQ ID NO: 119 - DNA, 18 bp, Artificial Sequence
  ADHFE1 probe 7
caacaacactcacaccat

SEQ ID NO: 120 - DNA, 25 bp, Artificial Sequence
  ADHFE1 probe 8
taaataatacaaacaccactaaaac

SEQ ID NO: 121 - DNA, 26 bp, Artificial Sequence
  ADHFE1 probe 9
atacaaacaccactaaaacaactaac

SEQ ID NO: 122 - DNA, 25 bp, Artificial Sequence
  ADHFE1 probe 10
actcaaaaccattttcccacgaaat

SEQ ID NO: 123 - DNA, 27 bp, Artificial Sequence
  ADHFE1 probe 11
aacgaaaaacgccactacccgatacga

SEQ ID NO: 124 - DNA, 28 bp, Artificial Sequence
  ADHFE1 probe 12
aacgccactacccgatacgaactacacc

SEQ ID NO: 125 - DNA, 25 bp, Artificial Sequence
  ADHFE1 probe 13
aaaaaccaaaacgccaactacccca

SEQ ID NO: 126 - DNA, 28 bp, Artificial Sequence
  ADHFE1 probe 14
cccacgaaataaaaaccaaaacgccaac

SEQ ID NO: 127 - DNA, 24 bp, Artificial Sequence
  ADHFE1 probe 15
caaaacgccaactaccccaacgac

SEQ ID NO: 128 - DNA, 16 bp, Artificial Sequence
  PPP2R5C probe 1
cgaaccgcgctctccc

SEQ ID NO: 129 - DNA, 21 bp, Artificial Sequence
  PPP2R5C probe 2
tttcctttccgtcccgtctcg

SEQ ID NO: 130 - DNA, 20 bp, Artificial Sequence
  PPP2R5C probe 3
aattaaaacgcgcaacgcaa

SEQ ID NO: 131 - DNA, 16 bp, Artificial Sequence
  PPP2R5C probe 4
cgattcgcgaacgacc

SEQ ID NO: 132 - DNA, 20 bp, Artificial Sequence
  PPP2R5C probe 5
ctttaccccgacctccgcta

SEQ ID NO: 133 - DNA, 16 bp, Artificial Sequence
  PPP2R5C probe 6
caaaccacactctccc

SEQ ID NO: 134 - DNA, 21 bp, Artificial Sequence
  PPP2R5C probe 7
tttcctttccatcccatctca

SEQ ID NO: 135 - DNA, 20 bp, Artificial Sequence
  PPP2R5C probe 8
aattaaaacacacaacacaa

SEQ ID NO: 136 - DNA, 20 bp, Artificial Sequence
  PPP2R5C probe 9
acacaattcacaaacaacca

SEQ ID NO: 137 - DNA, 20 bp, Artificial Sequence
  PPP2R5C probe 10
ctttaccccaacctccacta

SEQ ID NO: 138 - DNA, 19 bp, Artificial Sequence
  PPP2R5C probe 11
ccgcccgcgaaccgcgctc

SEQ ID NO: 139 - DNA, 28 bp, Artificial Sequence
  PPP2R5C probe 12
tacgcgctccaaccctctacttaaccgc

SEQ ID NO: 140 - DNA, 26 bp, Artificial Sequence
  PPP2R5C probe 13
caaccctctacttaaccgcccgcgaa

SEQ ID NO: 141 - DNA, 21 bp, Artificial Sequence
  PPP2R5C probe 14
cgttacgcgctccaaccctct

SEQ ID NO: 142 - DNA, 23 bp, Artificial Sequence
  PPP2R5C probe 15
tacgttacgcgctccaaccctct